European Patent Application EP 4 497 818 A1, published January 29, 2025. Title: Method for the fermentative production of L-lysine using C. glutamicum strains expressing heterologous nicotinamide nucleotide transhydrogenase PntAB. Applicant: Evonik Operations GmbH. Application EP. The sequence listing filed with the application follows.

SEQUENCE LISTING (12 sequences)

SEQ ID NO: 1 - DNA, 1533 bp, Escherichia coli
  source 1..1533: mol_type = genomic DNA
atgcgaattggcataccaagagaacggttaaccaatgaaacccgtgttgcagcaacgccaaaaacagtggaacagctgctgaaactgggttttaccgtcgcggtagagagcggcgcgggtcaactggcaagttttgacgataaagcgtttgtgcaagcgggcgctgaaattgtagaagggaatagcgtctggcagtcagagatcattctgaaggtcaatgcgccgttagatgatgaaattgcgttactgaatcctgggacaacgctggtgagttttatctggcctgcgcagaatccggaattaatgcaaaaacttgcggaacgtaacgtgaccgtgatggcgatggactctgtgccgcgtatctcacgcgcacaatcgctggacgcactaagctcgatggcgaacatcgccggttatcgcgccattgttgaagcggcacatgaatttgggcgcttctttaccgggcaaattactgcggccgggaaagtgccaccggcaaaagtgatggtgattggtgcgggtgttgcaggtctggccgccattggcgcagcaaacagtctcggcgcgattgtgcgtgcattcgacacccgcccggaagtgaaagaacaagttcaaagtatgggcgcggaattcctcgagctggattttaaagaggaagctggcagcggcgatggctatgccaaagtgatgtcggacgcgttcatcaaagcggaaatggaactctttgccgcccaggcaaaagaggtcgatatcattgtcaccaccgcgcttattccaggcaaaccagcgccgaagctaattacccgtgaaatggttgactccatgaaggcgggcagtgtgattgtcgacctggcagcccaaaacggcggcaactgtgaatacaccgtgccgggtgaaatcttcactacggaaaatggtgtcaaagtgattggttataccgatcttccgggccgtctgccgacgcaatcctcacagctttacggcacaaacctcgttaatctgctgaaactgttgtgcaaagagaaagacggcaatatcactgttgattttgatgatgtggtgattcgcggcgtgaccgtgatccgtgcgggcgaaattacctggccggcaccgccgattcaggtatcagctcagccgcaggcggcacaaaaagcggcaccggaagtgaaaactgaggaaaaatgtacctgctcaccgtggcgtaaatacgcgttgatggcgctggcaatcattctttttggctggatggcaagcgttgcgccgaaagaattccttgggcacttcaccgttttcgcgctggcctgcgttgtcggttattacgtggtgtggaatgtatcgcacgcgctgcatacaccgttgatgtcggtcaccaacgcgatttcagggattattgttgtcggagcactgttgcagattggccagggcggctgggttagcttccttagttttatcgcggtgcttatagccagcattaatattttcggtggcttcaccgtgactcagcgcatgctgaaaatgttccgcaaaaattaa

SEQ ID NO: 2 - DNA, 1389 bp, Escherichia coli
  source 1..1389: mol_type = genomic DNA
atgtctggaggattagttacagctgcatacattgttgccgcgatcctgtttatcttcagtctggccggtctttcgaaacatgaaacgtctcgccagggtaacaacttcggtatcgccgggatggcgattgcgttaatcgcaaccatttttggaccggatacgggtaatgttggctggatcttgctggcgatggtcattggtggggcaattggtatccgtctggcgaagaaagttgaaatgaccgaaatgccagaactggtggcgatcctgcatagcttcgtgggtctggcggcagtgctggttggctttaacagctatctgcatcatgacgcgggaatggcaccgattctggtcaatattcacctgacggaagtgttcctcggtatcttcatcggggcggtaacgttcacgggttcggtggtggcgttcggcaaactgtgtggcaagatttcgtctaaaccattgatgctgccaaaccgtcacaaaatgaacctggcggctctggtcgtttccttcctgctgctgattgtatttgttcgcacggacagcgtcggcctgcaagtgctggcattgctgataatgaccgcaattgcgctggtattcggctggcatttagtcgcctccatcggtggtgcagatatgccagtggtggtgtcgatgctgaactcgtactccggctgggcggctgcggctgcgggctttatgctcagcaacgacctgctgattgtgaccggtgcgctggtcggttcttcgggggctatcctttcttacattatgtgtaaggcgatgaaccgttcctttatcagcgttattgcgggtggtttcggcaccgacggctcttctactggcgatgatcaggaagtgggtgagcaccgcgaaatcaccgcagaagagacagcggaactgctgaaaaactcccattcagtgatcattactccggggtacggcatggcagtcgcgcaggcgcaatatcctgtcgctgaaattactgagaaattgcgcgctcgtggtattaatgtgcgtttcggtatccacccggtcgcggggcgtttgcctggacatatgaacgtattgctggctgaagcaaaagtaccgtatgacatcgtgctggaaatggacgagatcaatgatgactttgctgataccgataccgtactggtgattggtgctaacgatacggttaacccggcggcgcaggatgatccgaagagtccgattgctggtatgcctgtgctggaagtgtggaaagcgcagaacgtgattgtctttaaacgttcgatgaacactggctatgctggtgtgcaaaacccgctgttcttcaaggaaaacacccacatgctgtttggtgacgccaaagccagcgtggatgcaatcctgaaagctctgtaa

SEQ ID NO: 3 - protein, 510 aa, Escherichia coli
MRIGIPRERLTNETRVAATPKTVEQLLKLGFTVAVESGAGQLASFDDKAFVQAGAEIVEGNSVWQSEIILKVNAPLDDEIALLNPGTTLVSFIWPAQNPELMQKLAERNVTVMAMDSVPRISRAQSLDALSSMANIAGYRAIVEAAHEFGRFFTGQITAAGKVPPAKVMVIGAGVAGLAAIGAANSLGAIVRAFDTRPEVKEQVQSMGAEFLELDFKEEAGSGDGYAKVMSDAFIKAEMELFAAQAKEVDIIVTTALIPGKPAPKLITREMVDSMKAGSVIVDLAAQNGGNCEYTVPGEIFTTENGVKVIGYTDLPGRLPTQSSQLYGTNLVNLLKLLCKEKDGNITVDFDDVVIRGVTVIRAGEITWPAPPIQVSAQPQAAQKAAPEVKTEEKCTCSPWRKYALMALAIILFGWMASVAPKEFLGHFTVFALACVVGYYVVWNVSHALHTPLMSVTNAISGIIVVGALLQIGQGGWVSFLSFIAVLIASINIFGGFTVTQRMLKMFRKN

SEQ ID NO: 4 - protein, 462 aa, Escherichia coli
MSGGLVTAAYIVAAILFIFSLAGLSKHETSRQGNNFGIAGMAIALIATIFGPDTGNVGWILLAMVIGGAIGIRLAKKVEMTEMPELVAILHSFVGLAAVLVGFNSYLHHDAGMAPILVNIHLTEVFLGIFIGAVTFTGSVVAFGKLCGKISSKPLMLPNRHKMNLAALVVSFLLLIVFVRTDSVGLQVLALLIMTAIALVFGWHLVASIGGADMPVVVSMLNSYSGWAAAAAGFMLSNDLLIVTGALVGSSGAILSYIMCKAMNRSFISVIAGGFGTDGSSTGDDQEVGEHREITAEETAELLKNSHSVIITPGYGMAVAQAQYPVAEITEKLRARGINVRFGIHPVAGRLPGHMNVLLAEAKVPYDIVLEMDEINDDFADTDTVLVIGANDTVNPAAQDDPKSPIAGMPVLEVWKAQNVIVFKRSMNTGYAGVQNPLFFKENTHMLFGDAKASVDAILKAL

SEQ ID NO: 5 - DNA, 1554 bp, Corynebacterium urealyticum
  source 1..1554: mol_type = genomic DNA
gtgcgtatcggtattccggttgagccgggtgagaaccagccgctggtggcagccacaccagacacggtcggcaagctcatcaagcttggctatgacgttgaagtacaggcaggtgccggcgaagacgccgcctaccctgacgccctctaccgcgaggccggcgcgagcatcgtaggcgaggaggtctgggaagcggacatcgtcacgacgctcgacaccccgcccaaggagaagcgcgacctcatgcgctccggagccaccctgatctgccgcatggctccaggccgcaacgaggagctcatcaacgagctcgccaaccgtggcatcaccgggctcgcgatggacgctgtgccgcgtatttcccgcgcacagtccatggatgtcctctcctccatggcaaacatcgccggctaccgcgcagtcatcgaggccgccaacgccttcggtcgactgttcaccggccaggtcaccgcggcaggtaaggtgccgccggcaaaggtctacgtcatcggcgctggtgtcgctggcctggccgcgatcggtaccgccaactccatgggcgcgatcgtcaaggccaccgacctgcgcgtcgaggcaggcgagcaggtcgagtccatgggggcggaattcgtcgccatccaggaagaggccgagaagtccgaggacggctacgccaaggagatgacccaagaccaggcggaactcgctgcgaagatctattcccagcagtccgccgaagccgacatcgtcatcaccaccgcaaacattccgggccgcacctcgccggtgctgctcaccgaggaagatgtcgccaacatgcgtccgggcagcgtcgtcgtcgacctggcggcagccaacggtggtaactgcgcgctgacgaagccgggcgaggtcttcgtcaccgataacggcgtgaccatcattggctacaccgacctggcgggccgcctgcctggccaggcctcccagctgttcggccagaacatcgtcaacctgttcaagctgatcacgccggagaaggacggccagcgcgtgctggacctggatgacgagatcatccgcaccatcaccgtcaccctcaatgacggccaggagacctccgtcctctggccgccaccaccggtgagcgtgtccgtcgccccgcagcagcagcccgcgcaggacacgcaggccgccgaggagccggagaagcaagccttcatgggtggccccttcgccaagatcggtctggccatcgccatcctactgggcgctgcaatcgtcctggtcagcccgctgggaatgagcggcaacttcgtcgtcctgaccctggccatcgtgctgggcttctacgtgatctccgctgtcaccccgaccctgcacaccccgttgatgtccgagacgaacgcgatttcaggaatcgtcctggtcggcgcgatcttgcaggtcaacagccccaatatcatcgttacggtcctcgcgttcctggcaatcgtcgtgtcctccgtcaacgtgttcggtggcttcgccatcacagaccgcatgctcggcatgttcgttaaggaggatgcataa

SEQ ID NO: 6 - DNA, 1488 bp, Corynebacterium urealyticum
  source 1..1488: mol_type = genomic DNA
atgactgccactctgattctttcgcaggcagcgaccggcgagaacgccacgctgctggattggctggcccggatctcgaacctggcctacatcgtggctgccgtgctcttcctcatggcactggccggcctctctaagccggagaccgcaaagcgcggtaacacgctgggcatgagcggtatggctgttgccatcgccgtggccatcttccaggccgtggttcactccaccaccgattccgatgccctggacccggtcatcaccgtcgtcctcattgccctggctatgagcctcggtgcggcctacggcatcaagcgcgcgcactccgtcgagatgactggtctgccgcagctgatcgcgctgttcaacggcatggtcggtctgggcgcggtcttcatcggctacaactccttcgtttccgagtccgccgactcgatgggtgctgccgcctacaacttccacctgggtgaggtcttcctcggcatcttcatcggtgccgtgaccttcaccggctcgatcctggctggcctgaagctctccggcaaggtcaagggcgccccgctgctgctgccggcccgtaacctgctgaacgtcgccatcctggtgatcagcctcgtgctcatggtcgtgttcatcctcgcgggtgaaggcaccaccgcctggatcgcggttggcatcatgaccgccctggcgctgttcatgggctggcacctggtcgctgccattggcggtggcgacatgccggtcgtcgtgtccatcatgaactcctactccggctgggcagctgccttcaccggtctgatgctgcagaacccgctgctgatcatcaccggtgcgctggtcggttcctccggtgcattcctctcctacgtgatgtgccaggcgatgaaccgctccttcctgaacgtcctgctgggcggcttcggcaccgacggtggcgcggtcgcggagggtgtcgacggcacccacaccgagatcgacaccgacgaggctgtcgcgatgctcaaggacgcgaagaacatcatgatcaccccgggctacggcatggctgtctcccaagcgcagtacacggtcgctgagctgacccgcaagctgcgcgaccagggtaagactgtccagttcggtatccacccggtcgccggtcgcctgcctggccacatgaacgtcctgctggctgaggcgaaggtcccttatgacatcgtcatggatatggaggagatcaacgacgacttcgacgaggtcgacgtggtcctggtcatcggcgcgaacgatacggtcaacccgagcgctgagatgccgggctccccgatcgccggcatgccggttctgaaggtgtgggaggctgagcgcgtgatcgtgctgaagcgttccatgggtgccggttactccggtgcgcagaacccgctgttcttcaacgagaacaccgacatgctgctcggtgatgcgaaggcatccatcgagaagctggccgcagggatcagcaactaa

SEQ ID NO: 7 - protein, 517 aa, Corynebacterium urealyticum
MRIGIPVEPGENQPLVAATPDTVGKLIKLGYDVEVQAGAGEDAAYPDALYREAGASIVGEEVWEADIVTTLDTPPKEKRDLMRSGATLICRMAPGRNEELINELANRGITGLAMDAVPRISRAQSMDVLSSMANIAGYRAVIEAANAFGRLFTGQVTAAGKVPPAKVYVIGAGVAGLAAIGTANSMGAIVKATDLRVEAGEQVESMGAEFVAIQEEAEKSEDGYAKEMTQDQAELAAKIYSQQSAEADIVITTANIPGRTSPVLLTEEDVANMRPGSVVVDLAAANGGNCALTKPGEVFVTDNGVTIIGYTDLAGRLPGQASQLFGQNIVNLFKLITPEKDGQRVLDLDDEIIRTITVTLNDGQETSVLWPPPPVSVSVAPQQQPAQDTQAAEEPEKQAFMGGPFAKIGLAIAILLGAAIVLVSPLGMSGNFVVLTLAIVLGFYVISAVTPTLHTPLMSETNAISGIVLVGAILQVNSPNIIVTVLAFLAIVVSSVNVFGGFAITDRMLGMFVKEDA

SEQ ID NO: 8 - protein, 495 aa, Corynebacterium urealyticum
MTATLILSQAATGENATLLDWLARISNLAYIVAAVLFLMALAGLSKPETAKRGNTLGMSGMAVAIAVAIFQAVVHSTTDSDALDPVITVVLIALAMSLGAAYGIKRAHSVEMTGLPQLIALFNGMVGLGAVFIGYNSFVSESADSMGAAAYNFHLGEVFLGIFIGAVTFTGSILAGLKLSGKVKGAPLLLPARNLLNVAILVISLVLMVVFILAGEGTTAWIAVGIMTALALFMGWHLVAAIGGGDMPVVVSIMNSYSGWAAAFTGLMLQNPLLIITGALVGSSGAFLSYVMCQAMNRSFLNVLLGGFGTDGGAVAEGVDGTHTEIDTDEAVAMLKDAKNIMITPGYGMAVSQAQYTVAELTRKLRDQGKTVQFGIHPVAGRLPGHMNVLLAEAKVPYDIVMDMEEINDDFDEVDVVLVIGANDTVNPSAEMPGSPIAGMPVLKVWEAERVIVLKRSMGAGYSGAQNPLFFNENTDMLLGDAKASIEKLAAGISN

SEQ ID NO: 9 - DNA, 4726 bp, synthetic construct
  source 1..4726: mol_type = other DNA
cccggggcttcacgggcggcgtcagttaacttcacattcacaccgttaagcctatgcgttggggtaaaaattatggcagattggtgcttaagtaatggactgttttcaccctttaaacttctagatttaaacacgaggggtttcggtagcacggtttagtaacttgtcaaaggcttgcaaatacccactgctactactctgatggcgattaagcgaactttactatgactcgaaaatttagaagactccacgatctcggatatttcatcattccgtttgttgaatttttaagtattgcggcaggatactttcttattaaaactgcagcggatgagtttggaaagcttaattttatcgggacgattctcgtagtcggaggggtcgtttccctgtttaccgggtggccacttctattcgcaagagtgaatgattttaggtgggatgcagtttaccttgtgggtggagcggtatttttagcattcctttttctggggccaaaggaaatgacagttcttggactggtggcgatgtttgctggtccgggaatgctaatagcagggttttcatatctgagtcgtcgtattattgcgtattttgtggaattgaggcggttgcaacctagtgattaagaggctgtgatcacaccatggcttgaagtaaatggagaacagcttgaagcgccacaaatgctcatacggtgtctgcaagaaagacatttgtaaagctgctggtagcccaggtaaaaaatgaaatcactgcaatgcgtggatagtcctgggaaatatgctcacagtggcggttgaatttggggggtttatttcattcactttggcttgaagtcgtgcaggtcaggggagtgttgcccgaaaacattgagaggaaaacaaaaaccgatgtttgattgggggaatcgtgtggtataatggtaggacgcagtgactgctatcacccttggcggtctcttgttgaaaggaataattactctaatgcgaatcggcatcccgcgcgaacgtctgactaatgagacccgtgtcgctgctaccccaaagaccgtcgaacagctgctgaagctcggcttcaccgttgcagtggagtccggcgccggacagctcgcgtccttcgatgacaaggctttcgtgcaggcaggcgcagagatcgttgagggcaactctgtctggcagtccgagatcattctcaaggtcaacgccccactggacgacgaaatcgcgttgctcaacccaggcaccaccctggtttccttcatctggcccgctcagaatccagagctcatgcaaaagctggcagagcgtaacgtgactgttatggccatggactctgtcccacgtatctcccgcgctcagtccctcgacgcactgtccagcatggccaacatcgctggctaccgcgcaatcgtcgaggcagcacacgagttcggccgcttctttaccggccagatcacagctgcaggaaaggtccctcctgcaaaagttatggttatcggtgcaggcgtagctggacttgcagcaatcggcgcagcaaactccctcggcgctatcgtccgtgcgtttgacactcgcccagaagttaaggaacaggtccagagcatgggcgctgaattcctggagctggacttcaaggaagaagcaggctccggcgacggctacgcaaaggtcatgtccgacgctttcatcaaggcagaaatggagctgttcgcagcacaggcaaaggaggtagacatcatcgttaccaccgcgctcatcccaggaaagccggcaccaaagctcatcacccgcgaaatggtcgacagcatgaaggcaggctccgtcatcgtcgaccttgcagcacaaaacggtggcaactgcgaatacacggttcctggtgagatcttcaccaccgaaaacggcgtgaaggtgatcggctacactgacctgccaggtcgtttgcctacccaatcctctcagctgtacggaaccaacctggtcaacctcctgaagctgctgtgcaaggaaaaggacggcaacatcaccgtcgacttcgacgatgttgtcattcgtggtgttactgtgattcgcgccggcgaaatcacctggcccgctccaccaatccaggtatctgcacagccacaggctgcccagaaggcagcaccagaggtgaagaccgaggaaaagtgcacctgctcaccatggcgcaaatacgcactcatggcactcgctatcatcctcttcggctggatggcgtccgtcgcaccaaaggagttcctgggccacttcaccgttttcgctctcgcttgcgtagttggctactacgttgtgtggaacgtttcccacgctctgcacactccactgatgtccgtcaccaacgccatctccggaatcattgttgtaggcgccctcctgcagatcggccagggcggttgggtttccttcctctccttcatcgctgtgttgatcgcctccatcaacatcttcggtggcttcacggtaacccagcgcatgctgaagatgttccgcaagaactaaggggtaacatatgtccggtggccttgttaccgcagcatacatcgtcgccgccatcctgttcatcttctctctggccggcctctccaagcacgaaacttcccgtcagggcaacaacttcggcatcgctggtatggcaatcgcactgatcgccaccatctttggaccggacaccggcaacgttggctggattctgctcgcaatggtgatcggcggcgccatcggcatccgccttgctaagaaggtcgaaatgaccgaaatgccagagctcgttgctattctccactcattcgtcggtctggctgcagttctggtaggattcaactcttacctgcaccacgatgcaggtatggcaccaatcctggtgaacatccacctcaccgaagttttcttgggcatcttcatcggcgctgttaccttcaccggctctgttgtcgcatttggtaagctgtgcggtaagatctcctccaagccactcatgctgccaaaccgccacaagatgaacctagcagcactggtcgtctcttttctccttctcatcgttttcgtgcgtaccgattccgtcggactgcaggtccttgctcttttgatcatgaccgccatcgcactcgttttcggctggcacctcgtagcctccatcggcggcgctgacatgccagttgtcgtcagcatgctgaactcctactccggctgggctgcagctgccgcaggcttcatgctgtccaacgatctccttatcgttaccggcgcgctggtgggctcctccggtgcaattctcagctacatcatgtgcaaggccatgaaccgctccttcatctccgtcatcgcaggcggcttcggaaccgatggctcctccaccggcgacgaccaggaagttggcgagcaccgcgaaatcaccgccgaagagaccgctgagcttcttaagaactcccactccgtcatcattaccccaggctacggtatggccgtcgcacaggcacagtacccagtcgccgaaatcacagaaaagcttcgcgcgcgtggcatcaacgttcgcttcggcatccacccagtcgcaggccgactcccaggacacatgaacgttctgctggcagaggctaaggtgccatacgatatcgttttggagatggacgaaattaacgacgacttcgcagacaccgataccgtactggttatcggcgcaaacgacactgtgaacccagccgcacaagacgacccaaagtcccctatcgcaggaatgccagtcctggaagtctggaaggcccagaacgtgatcgttttcaagcgaagcatgaacaccggatacgctggcgttcagaacccactattcttcaaggaaaacacccacatgctcttcggcgatgctaaggcctccgttgacgcaattctcaaggctctctaataaacaaaagcgttgcgcgtgtggcattgaaagcggtggaactacctattggatatgagtgtgcttcactcccgaattcggtgatttggaatccaaactttaaagaaaaacaccgctgcccctccacctgcgcgaagcaggggaggggcagcggctgagaaaaatctggagcgtgttatctatgcagtgtctgggtttttagtgcacctttccttttcggatgtccttgttgaaaatgacaccggaagtaacatcctcatcaatctcctccaaggtacgtccacgagtttcaggaacctgggtgtagatgaagatcaaggcaaccacaccgattccggcgaacatgaagaaggttccggttagtcctactgcttccatgatggttgggaagaacaatccgaggaacgcgtttgcgatccagaggaagaacactgagataccgattgcgaaaccgcgcattgccagcgggaagagctcagagagcataacccaggtagctacgttgaggaaggtctgcatggatcccacgaagaccacaaccagagtcaagataacgtaggggcgaagaggatcgccgactgggaatgctacggatgcgataccgatcaatacgtggctaatggtggtgagagaataaccggtaatgagggtggtacggcggttgatacgatccatcatccacagtgcgatgaatgcaccgacaactgcgatcactcctggcgccacgttggcgatcagagctgcattctcggagaaaccagcctcaatgagaacaacctggccgtagtacatgatggagtcctgcagg

SEQ ID NO: 10 - DNA, 4839 bp, synthetic construct
  source 1..4839: mol_type = other DNA
tctagagcttcacgggcggcgtcagttaacttcacattcacaccgttaagcctatgcgttggggtaaaaattatggcagattggtgcttaagtaatggactgttttcaccctttaaacttcgagatttaaacacgaggggtttcggtagcacggtttagtaacttgtcaaaggcttgcaaatacccactgctactactctgatggcgattaagcgaactttactatgactcgaaaatttagaagactccacgatctcggatatttcatcattccgtttgttgaatttttaagtattgcggcaggatactttcttattaaaactgcagcggatgagtttggaaagcttaattttatcgggacgattctcgtagtcggaggggtcgtttccctgtttaccgggtggccacttctattcgcaagagtgaatgattttaggtgggatgcagtttaccttgtgggtggagcggtatttttagcattcctttttctggggccaaaggaaatgacagttcttggactggtggcgatgtttgctggtccgggaatgctaatagcagggttttcatatctgagtcgtcgtattattgcgtattttgtggaattgaggcggttgcaacctagtgattaagaggctgtgatcacaccatggcttgaagtaaatggagaacagcttgaagcgccacaaatgctcatacggtgtctgcaagaaagacatttgtaaagctgctggtagcccaggtaaaaaatgaaatcactgcaatgcgtggatagtcctgggaaatatgctcacagtggcggttgaatttggggggtttatttcattcactttggcttgaagtcgtgcaggtcaggggagtgttgcccgaaaacattgagaggaaaacaaaaaccgatgtttgattgggggaatcgtgtggtataatggtaggacgcagtgactgctatcacccttggcggtctcttgttgaaaggaataattactctaatgcgtatcggtattccggttgagccgggtgagaaccagccgctggtggcagccacaccagacacggtcggcaagctcatcaagcttggctatgacgttgaagtacaggcaggtgccggcgaagacgccgcctaccctgacgccctctaccgcgaggccggcgcgagcatcgtaggcgaggaggtctgggaagcggacatcgtcacgacgctcgacaccccgcccaaggagaagcgcgacctcatgcgctccggagccaccctgatctgccgcatggctccaggccgcaacgaggagctcatcaacgagctcgccaaccgtggcatcaccgggctcgcgatggacgctgtgccgcgtatttcccgcgcacagtccatggatgtcctctcctccatggcaaacatcgccggctaccgcgcagtcatcgaggccgccaacgccttcggtcgactgttcaccggccaggtcaccgcggcaggtaaggtgccgccggcaaaggtctacgtcatcggcgctggtgtcgctggcctggccgcgatcggtaccgccaactccatgggcgcgatcgtcaaggccaccgacctgcgcgtcgaggcaggcgagcaggtcgagtccatgggggcggaattcgtcgccatccaggaagaggccgagaagtccgaggacggctacgccaaggagatgacccaagaccaggcggaactcgctgcgaagatctattcccagcagtccgccgaagccgacatcgtcatcaccaccgcaaacattccgggccgcacctcgccggtgctgctcaccgaggaagatgtcgccaacatgcgtccgggcagcgtcgtcgtcgacctggcggcagccaacggtggtaactgcgcgctgacgaagccgggcgaggtcttcgtcaccgataacggcgtgaccatcattggctacaccgacctggcgggccgcctgcctggccaggcctcccagctgttcggccagaacatcgtcaacctgttcaagctgatcacgccggagaaggacggccagcgcgtgctggacctggatgacgagatcatccgcaccatcaccgtcaccctcaatgacggccaggagacctccgtcctctggccgccaccaccggtgagcgtgtccgtcgccccgcagcagcagcccgcgcaggacacgcaggccgccgaggagccggagaagcaagccttcatgggtggccccttcgccaagatcggtctggccatcgccatcctactgggcgctgcaatcgtcctggtcagcccgctgggaatgagcggcaacttcgtcgtcctgaccctggccatcgtgctgggcttctacgtgatctccgctgtcaccccgaccctgcacaccccgttgatgtccgagacgaacgcgatttcaggaatcgtcctggtcggcgcgatcttgcaggtcaacagccccaatatcatcgttacggtcctcgcgttcctggcaatcgtcgtgtcctccgtcaacgtgttcggtggcttcgccatcacagaccgcatgctcggcatgttcgttaaggaggatgcataaaccatgactgccactctgattctttcgcaggcagcgaccggcgagaacgccacgctgctggattggctggcccggatctcgaacctggcctacatcgtggctgccgtgctcttcctcatggcactggccggcctctctaagccggagaccgcaaagcgcggtaacacgctgggcatgagcggtatggctgttgccatcgccgtggccatcttccaggccgtggttcactccaccaccgattccgatgccctggacccggtcatcaccgtcgtcctcattgccctggctatgagcctcggtgcggcctacggcatcaagcgcgcgcactccgtcgagatgactggtctgccgcagctgatcgcgctgttcaacggcatggtcggtctgggcgcggtcttcatcggctacaactccttcgtttccgagtccgccgactcgatgggtgctgccgcctacaacttccacctgggtgaggtcttcctcggcatcttcatcggtgccgtgaccttcaccggctcgatcctggctggcctgaagctctccggcaaggtcaagggcgccccgctgctgctgccggcccgtaacctgctgaacgtcgccatcctggtgatcagcctcgtgctcatggtcgtgttcatcctcgcgggtgaaggcaccaccgcctggatcgcggttggcatcatgaccgccctggcgctgttcatgggctggcacctggtcgctgccattggcggtggcgacatgccggtcgtcgtgtccatcatgaactcctactccggctgggcagctgccttcaccggtctgatgctgcagaacccgctgctgatcatcaccggtgcgctggtcggttcctccggtgcattcctctcctacgtgatgtgccaggcgatgaaccgctccttcctgaacgtcctgctgggcggcttcggcaccgacggtggcgcggtcgcggagggtgtcgacggcacccacaccgagatcgacaccgacgaggctgtcgcgatgctcaaggacgcgaagaacatcatgatcaccccgggctacggcatggctgtctcccaagcgcagtacacggtcgctgagctgacccgcaagctgcgcgaccagggtaagactgtccagttcggtatccacccggtcgccggtcgcctgcctggccacatgaacgtcctgctggctgaggcgaaggtcccttatgacatcgtcatggatatggaggagatcaacgacgacttcgacgaggtcgacgtggtcctggtcatcggcgcgaacgatacggtcaacccgagcgctgagatgccgggctccccgatcgccggcatgccggttctgaaggtgtgggaggctgagcgcgtgatcgtgctgaagcgttccatgggtgccggttactccggtgcgcagaacccgctgttcttcaacgagaacaccgacatgctgctcggtgatgcgaaggcatccatcgagaagctggccgcagggatcagcaactaataaacaaaagcgttgcgcgtgtggcattgaaagcggtggaactacctattggatatgagtgtgcttcactcccgaattcggtgatttggaatccaaactttaaagaaaaacaccgctgcccctccacctgcgcgaagcaggggaggggcagcggctgagaaaaatctggagcgtgttatctatgcagtgtctgggtttttagtgcacctttccttttcggatgtccttgttgaaaatgacaccggaagtaacatcctcatcaatctcctccaaggtacgtccacgagtttcaggaacctgggtgtagatgaagatcaaggcaaccacaccgattccggcgaacatgaagaaggttccggttagtcctactgcttccatgatggttgggaagaacaatccgaggaacgcgtttgcgatccagaggaagaacactgagataccgattgcgaaaccgcgcattgccagcgggaagagctcagagagcataacccaggtagctacgttgaggaaggtctgcatggatcccacgaagaccacaaccagagtcaagataacgtaggggcgaagaggatcgccgactgggaatgctacggatgcgataccgatcaatacgtggctaatggtggtgagagaataaccggtaatgagggtggtacggcggttgatacgatccatcatccacagtgcgatgaatgcaccgacaactgcgatcactcctggcgccacgttggcgatcagagctgcattctcggagaaaccagcctcaatgagaacaacctggccgtagtacatgatggagtcctgcagg

SEQ ID NO: 11 - DNA, 1266 bp, Corynebacterium glutamicum
  source 1..1266: mol_type = genomic DNA
  misc_feature 932: note = exchange of nucleobase cytosine (c) at position 932 to give thymine (t). The acc codon for threonine is thus altered to the atc codon for isoleucine.
gtggccctggtcgtacagaaatatggcggttcctcgcttgagagtgcggaacgcattagaaacgtcgctgaacggatcgttgccaccaagaaggctggaaatgatgtcgtggttgtctgctccgcaatgggagacaccacggatgaacttctagaacttgcagcggcagtgaatcccgttccgccagctcgtgaaatggatatgctcctgactgctggtgagcgtatttctaacgctctcgtcgccatggctattgagtcccttggcgcagaagcccaatctttcacgggctctcaggctggtgtgctcaccaccgagcgccacggaaacgcacgcattgttgatgtcactccaggtcgtgtgcgtgaagcactcgatgagggcaagatctgcattgttgctggtttccagggtgttaataaagaaacccgcgatgtcaccacgttgggtcgtggtggttctgacaccactgcagttgcgttggcagctgctttgaacgctgatgtgtgtgagatttactcggacgttgacggtgtgtataccgctgacccgcgcatcgttcctaatgcacagaagctggaaaagctcagcttcgaagaaatgctggaacttgctgctgttggctccaagattttggtgctgcgcagtgttgaatacgctcgtgcattcaatgtgccacttcgcgtacgctcgtcttatagtaatgatcccggcactttgattgccggctctatggaggatattcctgtggaagaagcagtccttaccggtgtcgcaaccgacaagtccgaagccaaagtaaccgttctgggtatttccgataagccaggcgaggctgcgaaggttttccgtgcgttggctgatgcagaaatcaacattgacatggttctgcagaacgtctcttctgtagaagacggcaccaccgacatcatcttcacctgccctcgttccgacggccgccgcgcgatggagatcttgaagaagcttcaggttcagggcaactggaccaatgtgctttacgacgaccaggtcggcaaagtctccctcgtgggtgctggcatgaagtctcacccaggtgttaccgcagagttcatggaagctctgcgcgatgtcaacgtgaacatcgaattgatttccacctctgagattcgtatttccgtgctgatccgtgaagatgatctggatgctgctgcacgtgcattgcatgagcagttccagctgggcggcgaagacgaagccgtcgtttatgcaggcaccggacgctaa

SEQ ID NO: 12 - protein, 421 aa, Corynebacterium glutamicum
  VARIANT 311: note = feedback resistant aspartokinase polypeptide variant LysC_T311I
MALVVQKYGGSSLESAERIRNVAERIVATKKAGNDVVVVCSAMGDTTDELLELAAAVNPVPPAREMDMLLTAGERISNALVAMAIESLGAEAQSFTGSQAGVLTTERHGNARIVDVTPGRVREALDEGKICIVAGFQGVNKETRDVTTLGRGGSDTTAVALAAALNADVCEIYSDVDGVYTADPRIVPNAQKLEKLSFEEMLELAAVGSKILVLRSVEYARAFNVPLRVRSSYSNDPGTLIAGSMEDIPVEEAVLTGVATDKSEAKVTVLGISDKPGEAAKVFRALADAEINIDMVLQNVSSVEDGTTDIIFTCPRSDGRRAMEILKKLQVQGNWTNVLYDDQVGKVSLVGAGMKSHPGVTAEFMEALRDVNVNIELISTSEIRISVLIREDDLDAAARALHEQFQLGGEDEAVVYAGTGR